European Patent Specification EP 3 880 364 B1, published April 17, 2024. Title: ANALYSIS SYSTEMS WITH MICROFLUIDIC DEVICES, MICROFLUIDIC DEVICES AND RELATED METHODS. Applicant: The University of North Carolina at Chapel Hill Henley, William Hampton Pfefferle, Adam D. Ramsey, John Michael Perkowski, Ellen Foot. The sequence listing filed with the application follows.

SEQUENCE LISTING (2 sequences)

SEQ ID NO: 1 - DNA, 49 bp, Artificial
  primer
aatacaatcataataatacaatatacatggartggctaaagacaagacc

SEQ ID NO: 2 - DNA, 25 bp, Artificial
  primer
tatattgtattattatgattgtatt